European Patent Specification EP 3 612 567 B1, published September 11, 2024. Title: ANTI-VTCN1 ANTIBODIES AND ANTIBODY DRUG CONJUGATES. Applicant: BLUEFIN BIOMEDICINE, INC. The sequence listing filed with the application follows.

SEQUENCE LISTING (308 sequences)

SEQ ID NO: 1 - protein, 119 aa, Artificial Sequence
  Description of Artificial Sequence: Synthetic polypeptide
QMQLKESGPGLVQPSQSLSITCTVSGFSLTSYGVQWVRQFSGKGLEWLGVIWSSGSTDYNAAFISRLSISKDNSKSQVFFKMNSLQPDDTAMYYCARDITTIVEGFAYWGQGTLVTVSA

SEQ ID NO: 2 - protein, 10 aa, Artificial Sequence
  Description of Artificial Sequence: Synthetic peptide
GFSLTSYGVQ

SEQ ID NO: 3 - protein, 16 aa, Artificial Sequence
  Description of Artificial Sequence: Synthetic peptide
VIWSSGSTDYNAAFIS

SEQ ID NO: 4 - protein, 10 aa, Artificial Sequence
  Description of Artificial Sequence: Synthetic peptide
ITTIVEGFAY

SEQ ID NO: 5 - protein, 108 aa, Artificial Sequence
  Description of Artificial Sequence: Synthetic polypeptide
IIVMTQSPKSMSMSVGERVTLSCKASENVGTYVSWYQQKPEQSPKLLIYGASNRYTGVPDRFTGSGSATDFTLTISSVQAEDLADYHCGQSYSYPFTFGSGTKLEIKR

SEQ ID NO: 6 - protein, 11 aa, Artificial Sequence
  Description of Artificial Sequence: Synthetic peptide
KASENVGTYVS

SEQ ID NO: 7 - protein, 7 aa, Artificial Sequence
  Description of Artificial Sequence: Synthetic peptide
GASNRYT

SEQ ID NO: 8 - protein, 9 aa, Artificial Sequence
  Description of Artificial Sequence: Synthetic peptide
GQSYSYPFT

SEQ ID NO: 9 - protein, 117 aa, Artificial Sequence
  Description of Artificial Sequence: Synthetic polypeptide
QIQLQESGPELKKPGETVKISCKASGYTFTTTGMQWVQKMPGKGFKWIGWINTHSGEPKYADDFKGRFAFSLETSASTAHLQISNLKNEDTATYFCARTSYWYLDVWGAGTTVTVSS

SEQ ID NO: 10 - protein, 10 aa, Artificial Sequence
  Description of Artificial Sequence: Synthetic peptide
GYTFTTTGMQ

SEQ ID NO: 11 - protein, 17 aa, Artificial Sequence
  Description of Artificial Sequence: Synthetic peptide
WINTHSGEPKYADDFKG

SEQ ID NO: 12 - protein, 7 aa, Artificial Sequence
  Description of Artificial Sequence: Synthetic peptide
SYWYLDV

SEQ ID NO: 13 - protein, 107 aa, Artificial Sequence
  Description of Artificial Sequence: Synthetic polypeptide
DIVMTQSQKFMSTSVGDRVSVTCKASQIVGTNIAWYQQKPGQSPKALIYSASYRNSGVPDRFTGSGSGTDFTLTITNVQSEDLAEYFCQQYNSYPLTFGAGTKLEIK

SEQ ID NO: 14 - protein, 11 aa, Artificial Sequence
  Description of Artificial Sequence: Synthetic peptide
KASQIVGTNIA

SEQ ID NO: 15 - protein, 7 aa, Artificial Sequence
  Description of Artificial Sequence: Synthetic peptide
SASYRNS

SEQ ID NO: 16 - protein, 9 aa, Artificial Sequence
  Description of Artificial Sequence: Synthetic peptide
QQYNSYPLT

SEQ ID NO: 17 - protein, 119 aa, Artificial Sequence
  Description of Artificial Sequence: Synthetic polypeptide
QIQLKESGPGLVQPSQSLSITCTVSGFSLTSYGVHWVRQSPGKGLEWLGVIWSGGYTDYNSAFISRLSISKDNSKSQVFFKMNSLQADDTAIYYCARDITTIVEGFAYWGQGTLVTVSA

SEQ ID NO: 18 - protein, 10 aa, Artificial Sequence
  Description of Artificial Sequence: Synthetic peptide
GFSLTSYGVH

SEQ ID NO: 19 - protein, 16 aa, Artificial Sequence
  Description of Artificial Sequence: Synthetic peptide
VIWSGGYTDYNSAFIS

SEQ ID NO: 20 - protein, 10 aa, Artificial Sequence
  Description of Artificial Sequence: Synthetic peptide
ITTIVEGFAY

SEQ ID NO: 21 - protein, 107 aa, Artificial Sequence
  Description of Artificial Sequence: Synthetic polypeptide
IIVMTQSPKSMSMSVGERITLNCKASENVGTYVSWYQQKPEQSPKLLIYGASNRYTGVPDHFTGSGSATDFTLTISSVQAEDLADYHCGQTYSYPFTFGSGTKLEIK

SEQ ID NO: 22 - protein, 11 aa, Artificial Sequence
  Description of Artificial Sequence: Synthetic peptide
KASENVGTYVS

SEQ ID NO: 23 - protein, 7 aa, Artificial Sequence
  Description of Artificial Sequence: Synthetic peptide
GASNRYT

SEQ ID NO: 24 - protein, 9 aa, Artificial Sequence
  Description of Artificial Sequence: Synthetic peptide
GQTYSYPFT

SEQ ID NO: 25 - protein, 119 aa, Artificial Sequence
  Description of Artificial Sequence: Synthetic polypeptide
EVQLQESGPGLVQPSQSLSITCTVSGFSLTSYGVHWVRQSPGKGLEWLGVIWSSGSTDYNAAFISRLSISKDNSKSQVFFKIHSLQADDTAIYYCARDITTIVEGFAYWAQGTLVTVSA

SEQ ID NO: 26 - protein, 10 aa, Artificial Sequence
  Description of Artificial Sequence: Synthetic peptide
GFSLTSYGVH

SEQ ID NO: 27 - protein, 16 aa, Artificial Sequence
  Description of Artificial Sequence: Synthetic peptide
VIWSSGSTDYNAAFIS

SEQ ID NO: 28 - protein, 10 aa, Artificial Sequence
  Description of Artificial Sequence: Synthetic peptide
ITTIVEGFAY

SEQ ID NO: 29 - protein, 107 aa, Artificial Sequence
  Description of Artificial Sequence: Synthetic polypeptide
NIVMTQSPKSMSMSVGERVTLICKASENVGTYVSWYQQKPEQSPKLLIYGASNRYTGVPDRFTGSGSATDFTLTISSVQAEDLADYHCGQTYSYPFTFGSGTKLEIK

SEQ ID NO: 30 - protein, 11 aa, Artificial Sequence
  Description of Artificial Sequence: Synthetic peptide
KASENVGTYVS

SEQ ID NO: 31 - protein, 7 aa, Artificial Sequence
  Description of Artificial Sequence: Synthetic peptide
GASNRYT

SEQ ID NO: 32 - protein, 9 aa, Artificial Sequence
  Description of Artificial Sequence: Synthetic peptide
GQTYSYPFT

SEQ ID NO: 33 - protein, 119 aa, Artificial Sequence
  Description of Artificial Sequence: Synthetic polypeptide
QIQLQESGPGLVQPSQSLSITCTVSGFSLTSYGVQWVRQSPGKGLEWLGVIWSGGSTDYNAAFISRLSISKDNSKSQVFFKMNSLQADDTAIYYCARDISTIVEGFAHWGQGTLVTVSS

SEQ ID NO: 34 - protein, 10 aa, Artificial Sequence
  Description of Artificial Sequence: Synthetic peptide
GFSLTSYGVQ

SEQ ID NO: 35 - protein, 16 aa, Artificial Sequence
  Description of Artificial Sequence: Synthetic peptide
VIWSGGSTDYNAAFIS

SEQ ID NO: 36 - protein, 10 aa, Artificial Sequence
  Description of Artificial Sequence: Synthetic peptide
ISTIVEGFAH

SEQ ID NO: 37 - protein, 107 aa, Artificial Sequence
  Description of Artificial Sequence: Synthetic polypeptide
NIVMTQSPKSMSMSVGERVTLSCKASEKVGTYVSWYQQKPEQSPKLLIYGASNRYTGVPDRFTGSGSATDFTLTISSVQAEDLADYHCGQSYRYPFTFGSGTKLEIK

SEQ ID NO: 38 - protein, 11 aa, Artificial Sequence
  Description of Artificial Sequence: Synthetic peptide
KASEKVGTYVS

SEQ ID NO: 39 - protein, 7 aa, Artificial Sequence
  Description of Artificial Sequence: Synthetic peptide
GASNRYT

SEQ ID NO: 40 - protein, 9 aa, Artificial Sequence
  Description of Artificial Sequence: Synthetic peptide
GQSYRYPFT

SEQ ID NO: 41 - protein, 117 aa, Artificial Sequence
  Description of Artificial Sequence: Synthetic polypeptide
QVQMKESGPELKKPGETVKISCKASGYTFTTTGMQWVQKMPGKGFKWIGWINTHSGEPKYADDFKGRFAFSLETSASTAHLQISNLKNEDTATYFCARTSYWYLDVWGAGTTVTVSS

SEQ ID NO: 42 - protein, 10 aa, Artificial Sequence
  Description of Artificial Sequence: Synthetic peptide
GYTFTTTGMQ

SEQ ID NO: 43 - protein, 17 aa, Artificial Sequence
  Description of Artificial Sequence: Synthetic peptide
WINTHSGEPKYADDFKG

SEQ ID NO: 44 - protein, 7 aa, Artificial Sequence
  Description of Artificial Sequence: Synthetic peptide
SYWYLDV

SEQ ID NO: 45 - protein, 107 aa, Artificial Sequence; identical to SEQ ID NO: 13
  Description of Artificial Sequence: Synthetic polypeptide

SEQ ID NO: 46 - protein, 11 aa, Artificial Sequence
  Description of Artificial Sequence: Synthetic peptide
KASQIVGTNIA

SEQ ID NO: 47 - protein, 7 aa, Artificial Sequence
  Description of Artificial Sequence: Synthetic peptide
SASYRNS

SEQ ID NO: 48 - protein, 9 aa, Artificial Sequence
  Description of Artificial Sequence: Synthetic peptide
QQYNSYPLT

SEQ ID NO: 49 - protein, 119 aa, Artificial Sequence
  Description of Artificial Sequence: Synthetic polypeptide
QIQLQESGPGLVQPSQSLSITCTVSGFSLTSYGVHWVRQSPGKGLEWLGVIWSSGSTDYNAAFISRLSISKDNSRSQVFFKMNSLQPDDTAIYYCARDITTIVEGFAYWAQGTLVTVSA

SEQ ID NO: 50 - protein, 10 aa, Artificial Sequence
  Description of Artificial Sequence: Synthetic peptide
GFSLTSYGVH

SEQ ID NO: 51 - protein, 16 aa, Artificial Sequence
  Description of Artificial Sequence: Synthetic peptide
VIWSSGSTDYNAAFIS

SEQ ID NO: 52 - protein, 10 aa, Artificial Sequence
  Description of Artificial Sequence: Synthetic peptide
ITTIVEGFAY

SEQ ID NO: 53 - protein, 107 aa, Artificial Sequence
  Description of Artificial Sequence: Synthetic polypeptide
NVVMTQSPKSMSMSVGERVTLICKASENVGTYVSWYQQKPEQSPKLLIYGASNRYTGVPDRFTGSGSATDFTLTISSVQAEDLADYHCGQTYSYPFAFGSGTKLEIK

SEQ ID NO: 54 - protein, 11 aa, Artificial Sequence
  Description of Artificial Sequence: Synthetic peptide
KASENVGTYVS

SEQ ID NO: 55 - protein, 7 aa, Artificial Sequence
  Description of Artificial Sequence: Synthetic peptide
GASNRYT

SEQ ID NO: 56 - protein, 9 aa, Artificial Sequence
  Description of Artificial Sequence: Synthetic peptide
GQTYSYPFA

SEQ ID NO: 57 - protein, 122 aa, Artificial Sequence
  Description of Artificial Sequence: Synthetic polypeptide
QVQLQESGPELVKPGASVKLSCKASGYIFTDYTIHWLKQSPGQGLEWIGWIYPGSGHTHYNDKFKGKATMTADKSSTTAYMQLSSLTSEDSAVFFCARGGESITTVFPLAYWGQGTLVTVSA

SEQ ID NO: 58 - protein, 10 aa, Artificial Sequence
  Description of Artificial Sequence: Synthetic peptide
GYIFTDYTIH

SEQ ID NO: 59 - protein, 17 aa, Artificial Sequence
  Description of Artificial Sequence: Synthetic peptide
WIYPGSGHTHYNDKFKG

SEQ ID NO: 60 - protein, 12 aa, Artificial Sequence
  Description of Artificial Sequence: Synthetic peptide
GESITTVFPLAY

SEQ ID NO: 61 - protein, 113 aa, Artificial Sequence
  Description of Artificial Sequence: Synthetic polypeptide
DIVMSQSPSSLAVSVGEKVTMSCKSSQSLLYSSDQKNYLAWYQQKPGQSPKLLIYWASTWESGVPDRFIGSGSGTDFTLTVSSVKAEDLAVYYCHQYYSYPPTFGAGTKLEIK

SEQ ID NO: 62 - protein, 17 aa, Artificial Sequence
  Description of Artificial Sequence: Synthetic peptide
KSSQSLLYSSDQKNYLA

SEQ ID NO: 63 - protein, 7 aa, Artificial Sequence
  Description of Artificial Sequence: Synthetic peptide
WASTWES

SEQ ID NO: 64 - protein, 9 aa, Artificial Sequence
  Description of Artificial Sequence: Synthetic peptide
HQYYSYPPT

SEQ ID NO: 65 - protein, 119 aa, Artificial Sequence
  Description of Artificial Sequence: Synthetic polypeptide
QVQLQQSGPGLVQPSQSLSITCTVSGFSLTSYGVHWVRQSPGKGLEWLGVIWSGGSTDYNAAFISRLSISKDNSKSQVFFKMNSLQADDTAIYYCARDITTIVEGFAYWGQGTLVTVSA

SEQ ID NO: 66 - protein, 10 aa, Artificial Sequence
  Description of Artificial Sequence: Synthetic peptide
GFSLTSYGVH

SEQ ID NO: 67 - protein, 16 aa, Artificial Sequence
  Description of Artificial Sequence: Synthetic peptide
VIWSGGSTDYNAAFIS

SEQ ID NO: 68 - protein, 10 aa, Artificial Sequence
  Description of Artificial Sequence: Synthetic peptide
ITTIVEGFAY

SEQ ID NO: 69 - protein, 107 aa, Artificial Sequence
  Description of Artificial Sequence: Synthetic polypeptide
NIVMTQSPKSMSMSVGERVTLSCKASENVGTYVSWYQQKPEQSPKLLIYGASNRYTGVPDRFTGSGSATDFTLTISSVQAEDVTDYHCGQTYSYPFTFGSGTKLEIK

SEQ ID NO: 70 - protein, 11 aa, Artificial Sequence
  Description of Artificial Sequence: Synthetic peptide
KASENVGTYVS

SEQ ID NO: 71 - protein, 7 aa, Artificial Sequence
  Description of Artificial Sequence: Synthetic peptide
GASNRYT

SEQ ID NO: 72 - protein, 9 aa, Artificial Sequence
  Description of Artificial Sequence: Synthetic peptide
GQTYSYPFT

SEQ ID NO: 73 - protein, 119 aa, Artificial Sequence
  Description of Artificial Sequence: Synthetic polypeptide
QIQLQQSGPGLVQPSQSLSITCTVSGFSLTSYGVQWVRQSPGKGLEWLGVIWSSGNTDYNAAFISRLTITKDNSKSQIFFKMNSLQADDTAIYYCARDITTIVEGFAYWGQGTLVTVSA

SEQ ID NO: 74 - protein, 10 aa, Artificial Sequence
  Description of Artificial Sequence: Synthetic peptide
GFSLTSYGVQ

SEQ ID NO: 75 - protein, 16 aa, Artificial Sequence
  Description of Artificial Sequence: Synthetic peptide
VIWSSGNTDYNAAFIS

SEQ ID NO: 76 - protein, 10 aa, Artificial Sequence
  Description of Artificial Sequence: Synthetic peptide
ITTIVEGFAY

SEQ ID NO: 77 - protein, 107 aa, Artificial Sequence
  Description of Artificial Sequence: Synthetic polypeptide
NIVMTQSPKSMSMSVGERVTLSCKASENVGTYVSWYQQKPEQSPKLLIYGASNRYTGVPDRFTGSGSATDFTLTISSVQAEDLADYHCGQTYSYPFTFGSGTKLEIK

SEQ ID NO: 78 - protein, 11 aa, Artificial Sequence
  Description of Artificial Sequence: Synthetic peptide
KASENVGTYVS

SEQ ID NO: 79 - protein, 7 aa, Artificial Sequence
  Description of Artificial Sequence: Synthetic peptide
GASNRYT

SEQ ID NO: 80 - protein, 9 aa, Artificial Sequence
  Description of Artificial Sequence: Synthetic peptide
GQTYSYPFT

SEQ ID NO: 81 - protein, 117 aa, Artificial Sequence
  Description of Artificial Sequence: Synthetic polypeptide
QIQLQQSGPELKKPGETVKISCKASGYTFTTAGMQWVQKMPGKGFKWLGWINTHSGEPKYADDFKGRFAFSLETSASTAYLQINNLKNEDTATYHCARTSYWYLDIWGAGTTVTVSS

SEQ ID NO: 82 - protein, 10 aa, Artificial Sequence
  Description of Artificial Sequence: Synthetic peptide
GYTFTTAGMQ

SEQ ID NO: 83 - protein, 17 aa, Artificial Sequence
  Description of Artificial Sequence: Synthetic peptide
WINTHSGEPKYADDFKG

SEQ ID NO: 84 - protein, 7 aa, Artificial Sequence
  Description of Artificial Sequence: Synthetic peptide
SYWYLDI

SEQ ID NO: 85 - protein, 107 aa, Artificial Sequence
  Description of Artificial Sequence: Synthetic polypeptide
DIVMTQSQKFMSTSVGDRVSVTCKASQNVGTNVAWYQQKPGQSPKALIYSASYRCSGVPDRFTGSGSGTDFTLTISNVQSEDLAEYFCQQYNSYPLTFGAGTKLEIK

SEQ ID NO: 86 - protein, 11 aa, Artificial Sequence
  Description of Artificial Sequence: Synthetic peptide
KASQNVGTNVA

SEQ ID NO: 87 - protein, 7 aa, Artificial Sequence
  Description of Artificial Sequence: Synthetic peptide
SASYRCS

SEQ ID NO: 88 - protein, 9 aa, Artificial Sequence
  Description of Artificial Sequence: Synthetic peptide
QQYNSYPLT

SEQ ID NO: 89 - protein, 123 aa, Artificial Sequence
  Description of Artificial Sequence: Synthetic polypeptide
QVQLQQPGAELVKPGASVKLSCKASGYSFTSYWMNWVKQRPGRGLEWIGRIHPSDSETHYNQNFKSKATLTVDKSSSTAYIQLNSLTSEDSAVYYCARPYYFYGSSPYAMDYWGQGASVTVSS

SEQ ID NO: 90 - protein, 10 aa, Artificial Sequence
  Description of Artificial Sequence: Synthetic peptide
GYSFTSYWMN

SEQ ID NO: 91 - protein, 17 aa, Artificial Sequence
  Description of Artificial Sequence: Synthetic peptide
RIHPSDSETHYNQNFKS

SEQ ID NO: 92 - protein, 13 aa, Artificial Sequence
  Description of Artificial Sequence: Synthetic peptide
YYFYGSSPYAMDY

SEQ ID NO: 93 - protein, 112 aa, Artificial Sequence
  Description of Artificial Sequence: Synthetic polypeptide
DVVMTQTPLSLPVSLGDQASISCRSSQSIVHSNGNTYLEWYLQKPGQSPKLLIYKVSNRFSGVPDRFSGSGSGTDFTFKISRVEAEDLGVYYCFQGSHVPYTFGGGTKLEIK

SEQ ID NO: 94 - protein, 16 aa, Artificial Sequence
  Description of Artificial Sequence: Synthetic peptide
RSSQSIVHSNGNTYLE

SEQ ID NO: 95 - protein, 7 aa, Artificial Sequence
  Description of Artificial Sequence: Synthetic peptide
KVSNRFS

SEQ ID NO: 96 - protein, 9 aa, Artificial Sequence
  Description of Artificial Sequence: Synthetic peptide
FQGSHVPYT

SEQ ID NO: 97 - protein, 119 aa, Artificial Sequence
  Description of Artificial Sequence: Synthetic polypeptide
QMQLQESGPGLVQPSQSLSITCTVSGFSLTSYGIHWVRQSPGKGLEWLGVIWSSGSTDYNAAFISRLSISKDNSKSQVFFKMNSLQSDDTAIHYCARDITTIAEGFAYWGQGTLVTVSS

SEQ ID NO: 98 - protein, 10 aa, Artificial Sequence
  Description of Artificial Sequence: Synthetic peptide
GFSLTSYGIH

SEQ ID NO: 99 - protein, 16 aa, Artificial Sequence
  Description of Artificial Sequence: Synthetic peptide
VIWSSGSTDYNAAFIS

SEQ ID NO: 100 - protein, 10 aa, Artificial Sequence
  Description of Artificial Sequence: Synthetic peptide
ITTIAEGFAY

SEQ ID NO: 101 - protein, 107 aa, Artificial Sequence
  Description of Artificial Sequence: Synthetic polypeptide
NIVMTQSPKSMSMSVGERVTLSCKASENVGTYVSWYQQKPEQSPKLLIYGASNRYTGVPDRFTGSGSATDFTLTISSVQAEDLADYHCGQSYSYPFTFGSGTKLEIK

SEQ ID NO: 102 - protein, 11 aa, Artificial Sequence
  Description of Artificial Sequence: Synthetic peptide
KASENVGTYVS

SEQ ID NO: 103 - protein, 7 aa, Artificial Sequence
  Description of Artificial Sequence: Synthetic peptide
GASNRYT

SEQ ID NO: 104 - protein, 9 aa, Artificial Sequence
  Description of Artificial Sequence: Synthetic peptide
GQSYSYPFT

SEQ ID NO: 105 - protein, 119 aa, Artificial Sequence
  Description of Artificial Sequence: Synthetic polypeptide
QVQLQQSGPGLVQPSQSLSITCTVSGFSLTSYGVQWVRQSPGKGLEWLGVIWSSGSTDYNAAFISRLSINKDNSKSQVFFKMNSLQPDDTAIYYCARDITTIVEGFAYWGQGTLVTVSA

SEQ ID NO: 106 - protein, 10 aa, Artificial Sequence
  Description of Artificial Sequence: Synthetic peptide
GFSLTSYGVQ

SEQ ID NO: 107 - protein, 16 aa, Artificial Sequence
  Description of Artificial Sequence: Synthetic peptide
VIWSSGSTDYNAAFIS

SEQ ID NO: 108 - protein, 10 aa, Artificial Sequence
  Description of Artificial Sequence: Synthetic peptide
ITTIVEGFAY

SEQ ID NO: 109 - protein, 107 aa, Artificial Sequence
  Description of Artificial Sequence: Synthetic polypeptide
IIVMTQSPKSMSMSVGERVTLSCKASENVGTYVSWYQQKPEQSPKLLIYGASNRYTGVPDRFTGSGSATDFTLTISSVQAEDLADYHCGQSYSYPFTFGSGTKLEIK

SEQ ID NO: 110 - protein, 11 aa, Artificial Sequence
  Description of Artificial Sequence: Synthetic peptide
KASENVGTYVS

SEQ ID NO: 111 - protein, 7 aa, Artificial Sequence
  Description of Artificial Sequence: Synthetic peptide
GASNRYT

SEQ ID NO: 112 - protein, 9 aa, Artificial Sequence
  Description of Artificial Sequence: Synthetic peptide
GQSYSYPFT

SEQ ID NO: 113 - protein, 119 aa, Artificial Sequence
  Description of Artificial Sequence: Synthetic polypeptide
QIQLQQSGPGLVQPSQSLSITCTVSGFSLTSYGVQWIRQSPGKGLEWLGVIWSSGSTDYNAAFLSRLSFSKDNSKSQVFFQMNSLQADDSAIYYCARDVTTIVEGFAHWGQGTLVTVSA

SEQ ID NO: 114 - protein, 10 aa, Artificial Sequence
  Description of Artificial Sequence: Synthetic peptide
GFSLTSYGVQ

SEQ ID NO: 115 - protein, 16 aa, Artificial Sequence
  Description of Artificial Sequence: Synthetic peptide
VIWSSGSTDYNAAFLS

SEQ ID NO: 116 - protein, 10 aa, Artificial Sequence
  Description of Artificial Sequence: Synthetic peptide
VTTIVEGFAH

SEQ ID NO: 117 - protein, 107 aa, Artificial Sequence
  Description of Artificial Sequence: Synthetic polypeptide
NIVMTQSPKSMSMSVGERVTLSCKASEKVGTYVSWYQQKPEQSPKLLIYGASNRYTGVPDRFTGSGSATDFTLTISSVQVEDLADYHCGQTYSYPFTFGSGTKLEIK

SEQ ID NO: 118 - protein, 11 aa, Artificial Sequence
  Description of Artificial Sequence: Synthetic peptide
KASEKVGTYVS

SEQ ID NO: 119 - protein, 7 aa, Artificial Sequence
  Description of Artificial Sequence: Synthetic peptide
GASNRYT

SEQ ID NO: 120 - protein, 9 aa, Artificial Sequence
  Description of Artificial Sequence: Synthetic peptide
GQTYSYPFT

SEQ ID NO: 121 - protein, 119 aa, Artificial Sequence
  Description of Artificial Sequence: Synthetic polypeptide
QIQLQESGPGLVQPSQSLSITCTVSGFSLTSYGVQWVRQSPGKGLEWLGVIWSSGSTDYNAAFISRLSISKDNSKSQVFFKMNSLQADDTAIYYCARDITTIVEGFAYWGQGTLVTVSA

SEQ ID NO: 122 - protein, 10 aa, Artificial Sequence
  Description of Artificial Sequence: Synthetic peptide
GFSLTSYGVQ

SEQ ID NO: 123 - protein, 16 aa, Artificial Sequence
  Description of Artificial Sequence: Synthetic peptide
VIWSSGSTDYNAAFIS

SEQ ID NO: 124 - protein, 10 aa, Artificial Sequence
  Description of Artificial Sequence: Synthetic peptide
ITTIVEGFAY

SEQ ID NO: 125 - protein, 107 aa, Artificial Sequence
  Description of Artificial Sequence: Synthetic polypeptide
NIVMTQSPKSMSMSVGERVTLRCKASENVNTYVSWYQQKPEQSPKLLIYGASNRYTGVPDRFTGSGSATDFTLTISSVQAEDLADYHCGQSYSYPFTFGSGTKLEIK

SEQ ID NO: 126 - protein, 11 aa, Artificial Sequence
  Description of Artificial Sequence: Synthetic peptide
KASENVNTYVS

SEQ ID NO: 127 - protein, 7 aa, Artificial Sequence
  Description of Artificial Sequence: Synthetic peptide
GASNRYT

SEQ ID NO: 128 - protein, 9 aa, Artificial Sequence
  Description of Artificial Sequence: Synthetic peptide
GQSYSYPFT

SEQ ID NO: 129 - protein, 119 aa, Artificial Sequence
  Description of Artificial Sequence: Synthetic polypeptide
QIQLKESGPGLVQPSQSLSITCTVSGFSLTSYGVQWVRQSPGKGLEWLGVIWSGGSTDYNAAFISRLSISKDNSKSQVFFKMNSLQADDTAIYYCARDITTIVEGFAYWAQGTLVTVSA

SEQ ID NO: 130 - protein, 10 aa, Artificial Sequence
  Description of Artificial Sequence: Synthetic peptide
GFSLTSYGVQ

SEQ ID NO: 131 - protein, 16 aa, Artificial Sequence
  Description of Artificial Sequence: Synthetic peptide
VIWSGGSTDYNAAFIS

SEQ ID NO: 132 - protein, 10 aa, Artificial Sequence
  Description of Artificial Sequence: Synthetic peptide
ITTIVEGFAY

SEQ ID NO: 133 - protein, 107 aa, Artificial Sequence; identical to SEQ ID NO: 77
  Description of Artificial Sequence: Synthetic polypeptide

SEQ ID NO: 134 - protein, 11 aa, Artificial Sequence
  Description of Artificial Sequence: Synthetic peptide
KASENVGTYVS

SEQ ID NO: 135 - protein, 7 aa, Artificial Sequence
  Description of Artificial Sequence: Synthetic peptide
GASNRYT

SEQ ID NO: 136 - protein, 9 aa, Artificial Sequence
  Description of Artificial Sequence: Synthetic peptide
GQTYSYPFT

SEQ ID NO: 137 - protein, 119 aa, Artificial Sequence
  Description of Artificial Sequence: Synthetic polypeptide
QVQLQQSGPGLVQPSQSLSITCTVSGFSLTSYGIHWVRQSPGKGLEWLGVIWSSGSTDYNAAFISRLSISKDNSKSQVFFKMNSLQSDDTAIHYCARDITTIAEGFAYWGQGTLVTVSA

SEQ ID NO: 138 - protein, 10 aa, Artificial Sequence
  Description of Artificial Sequence: Synthetic peptide
GFSLTSYGIH

SEQ ID NO: 139 - protein, 16 aa, Artificial Sequence
  Description of Artificial Sequence: Synthetic peptide
VIWSSGSTDYNAAFIS

SEQ ID NO: 140 - protein, 10 aa, Artificial Sequence
  Description of Artificial Sequence: Synthetic peptide
ITTIAEGFAY

SEQ ID NO: 141 - protein, 107 aa, Artificial Sequence; identical to SEQ ID NO: 101
  Description of Artificial Sequence: Synthetic polypeptide

SEQ ID NO: 142 - protein, 11 aa, Artificial Sequence
  Description of Artificial Sequence: Synthetic peptide
KASENVGTYVS

SEQ ID NO: 143 - protein, 7 aa, Artificial Sequence
  Description of Artificial Sequence: Synthetic peptide
GASNRYT

SEQ ID NO: 144 - protein, 9 aa, Artificial Sequence
  Description of Artificial Sequence: Synthetic peptide
GQSYSYPFT

SEQ ID NO: 145 - protein, 119 aa, Artificial Sequence
  Description of Artificial Sequence: Synthetic polypeptide
QVQMQESGPGLVQPSQSLSITCTVSGFSLTSYGVQWVRQSPGKGLQWLGVIWSSGSTDYNAAVISRLSISKDTSKSQVFFKMNSLQPDDTAIYYCARDITTIVEGFAYWGQGTLVTVSS

SEQ ID NO: 146 - protein, 10 aa, Artificial Sequence
  Description of Artificial Sequence: Synthetic peptide
GFSLTSYGVQ

SEQ ID NO: 147 - protein, 16 aa, Artificial Sequence
  Description of Artificial Sequence: Synthetic peptide
VIWSSGSTDYNAAVIS

SEQ ID NO: 148 - protein, 10 aa, Artificial Sequence
  Description of Artificial Sequence: Synthetic peptide
ITTIVEGFAY

SEQ ID NO: 149 - protein, 107 aa, Artificial Sequence; identical to SEQ ID NO: 109
  Description of Artificial Sequence: Synthetic polypeptide

SEQ ID NO: 150 - protein, 11 aa, Artificial Sequence
  Description of Artificial Sequence: Synthetic peptide
KASENVGTYVS

SEQ ID NO: 151 - protein, 7 aa, Artificial Sequence
  Description of Artificial Sequence: Synthetic peptide
GASNRYT

SEQ ID NO: 152 - protein, 9 aa, Artificial Sequence
  Description of Artificial Sequence: Synthetic peptide
GQSYSYPFT

SEQ ID NO: 153 - protein, 119 aa, Artificial Sequence
  Description of Artificial Sequence: Synthetic polypeptide
QIQLQQSGPGLVQPSQSLSITCTVSGFSLTSYGIHWVRQSPGKGLEWLGVIWSSGSTDYNAAFISRLSISKDNSKSQVFFKMNSLQSDDTAIHYCARDITTIAEGFAYWGQGTLVTVSA

SEQ ID NO: 154 - protein, 10 aa, Artificial Sequence
  Description of Artificial Sequence: Synthetic peptide
GFSLTSYGIH

SEQ ID NO: 155 - protein, 16 aa, Artificial Sequence
  Description of Artificial Sequence: Synthetic peptide
VIWSSGSTDYNAAFIS

SEQ ID NO: 156 - protein, 10 aa, Artificial Sequence
  Description of Artificial Sequence: Synthetic peptide
ITTIAEGFAY

SEQ ID NO: 157 - protein, 107 aa, Artificial Sequence; identical to SEQ ID NO: 101
  Description of Artificial Sequence: Synthetic polypeptide

SEQ ID NO: 158 - protein, 11 aa, Artificial Sequence
  Description of Artificial Sequence: Synthetic peptide
KASENVGTYVS

SEQ ID NO: 159 - protein, 7 aa, Artificial Sequence
  Description of Artificial Sequence: Synthetic peptide
GASNRYT

SEQ ID NO: 160 - protein, 9 aa, Artificial Sequence
  Description of Artificial Sequence: Synthetic peptide
GQSYSYPFT

SEQ ID NO: 161 - protein, 119 aa, Artificial Sequence
  Description of Artificial Sequence: Synthetic polypeptide
QVQLKQSGPGLVQPSQSLSITCTVSGFSLTSYGIHWVRQSPGKGLEWLGVIWSSGSTDYNAAFISRLSISKDNSKSQVFFKMNSLQSDDTAIHYCARDITTIAEGFAYWGQGTLVTVSA

SEQ ID NO: 162 - protein, 10 aa, Artificial Sequence
  Description of Artificial Sequence: Synthetic peptide
GFSLTSYGIH

SEQ ID NO: 163 - protein, 16 aa, Artificial Sequence
  Description of Artificial Sequence: Synthetic peptide
VIWSSGSTDYNAAFIS

SEQ ID NO: 164 - protein, 10 aa, Artificial Sequence
  Description of Artificial Sequence: Synthetic peptide
ITTIAEGFAY

SEQ ID NO: 165 - protein, 107 aa, Artificial Sequence; identical to SEQ ID NO: 101
  Description of Artificial Sequence: Synthetic polypeptide

SEQ ID NO: 166 - protein, 11 aa, Artificial Sequence
  Description of Artificial Sequence: Synthetic peptide
KASENVGTYVS

SEQ ID NO: 167 - protein, 7 aa, Artificial Sequence
  Description of Artificial Sequence: Synthetic peptide
GASNRYT

SEQ ID NO: 168 - protein, 9 aa, Artificial Sequence
  Description of Artificial Sequence: Synthetic peptide
GQSYSYPFT

SEQ ID NO: 169 - protein, 119 aa, Artificial Sequence
  Description of Artificial Sequence: Synthetic polypeptide
QIQLQESGPGLVQPSQSLSITCTVSGFSLTSYGVQWVRQSPGKGLEWLGVIWSGGSTDYNAAFISRLSISKDNSKSQVFFKMNSLQADDTAIYYCARDITTIVEGFAHWGQGTLVTVSA

SEQ ID NO: 170 - protein, 10 aa, Artificial Sequence
  Description of Artificial Sequence: Synthetic peptide
GFSLTSYGVQ

SEQ ID NO: 171 - protein, 16 aa, Artificial Sequence
  Description of Artificial Sequence: Synthetic peptide
VIWSGGSTDYNAAFIS

SEQ ID NO: 172 - protein, 10 aa, Artificial Sequence
  Description of Artificial Sequence: Synthetic peptide
ITTIVEGFAH

SEQ ID NO: 173 - protein, 107 aa, Artificial Sequence
  Description of Artificial Sequence: Synthetic polypeptide
NIVMTQSPKSMSMSVGERVTLSCKASEKVGTYVSWYQQKPEQSPKLLIYGASNRYTGVPDRFTGSGSATDFTLTISSVQAEDLADYHCGQSYSYPFTFGSGTKLEIK

SEQ ID NO: 174 - protein, 11 aa, Artificial Sequence
  Description of Artificial Sequence: Synthetic peptide
KASEKVGTYVS

SEQ ID NO: 175 - protein, 7 aa, Artificial Sequence
  Description of Artificial Sequence: Synthetic peptide
GASNRYT

SEQ ID NO: 176 - protein, 9 aa, Artificial Sequence
  Description of Artificial Sequence: Synthetic peptide
GQSYSYPFT

SEQ ID NO: 177 - protein, 122 aa, Artificial Sequence
  Description of Artificial Sequence: Synthetic polypeptide
QVQLQESGPELVKPGASVKLSCKASGYSFTDYTMHWVKQSPGQGLEWIGWIYPGSGNTMYNDKFKGEATMTADKSSSTTYMQLSSLTSEDSAVYFCARGGDSIITVFPFTYWGQGTLVTVSA

SEQ ID NO: 178 - protein, 10 aa, Artificial Sequence
  Description of Artificial Sequence: Synthetic peptide
GYSFTDYTMH

SEQ ID NO: 179 - protein, 24 aa, Artificial Sequence
  Description of Artificial Sequence: Synthetic peptide
WIYPGSGNTMYNDKFKGEATMTAD

SEQ ID NO: 180 - protein, 12 aa, Artificial Sequence
  Description of Artificial Sequence: Synthetic peptide
GDSIITVFPFTY

SEQ ID NO: 181 - protein, 113 aa, Artificial Sequence
  Description of Artificial Sequence: Synthetic polypeptide
DIVMSQSPSSLAVSVGEKVTMSCKSSQSLLYSSNQKNYLAWYQQKPGQSPELLIYWASTRESGVPDRFTGSGSGTDFTLTISSVKAEDLAVYYCQQYYSYPPTFGAGTKLEIK

SEQ ID NO: 182 - protein, 17 aa, Artificial Sequence
  Description of Artificial Sequence: Synthetic peptide
KSSQSLLYSSNQKNYLA

SEQ ID NO: 183 - protein, 7 aa, Artificial Sequence
  Description of Artificial Sequence: Synthetic peptide
WASTRES

SEQ ID NO: 184 - protein, 9 aa, Artificial Sequence
  Description of Artificial Sequence: Synthetic peptide
QQYYSYPPT

SEQ ID NO: 185 - protein, 282 aa, Homo sapiens
MASLGQILFWSIISIIIILAGAIALIIGFGISGRHSITVTTVASAGNIGEDGILSCTFEPDIKLSDIVIQWLKEGVLGLVHEFKEGKDELSEQDEMFRGRTAVFADQVIVGNASLRLKNVQLTDAGTYKCYIITSKGKGNANLEYKTGAFSMPEVNVDYNASSETLRCEAPRWFPQPTVVWASQVDQGANFSEVSNTSFELNSENVTMKVVSVLYNVTINNTYSCMIENDIAKATGDIKVTESEIKRRSHLQLLNSKASLCVSSFFAISWALLPLSPYLMLK

SEQ ID NO: 186 - DNA, 40 bp, Artificial Sequence
  Description of Artificial Sequence: Synthetic primer
atagctcttcagggaccatgaarcayctgtggttcttcct

SEQ ID NO: 187 - DNA, 39 bp, Artificial Sequence
  Description of Artificial Sequence: Synthetic primer
atagctcttcagggaccatggacatactttgttccacgc

SEQ ID NO: 188 - DNA, 39 bp, Artificial Sequence
  Description of Artificial Sequence: Synthetic primer
atagctcttcagggaccatggacacactttgctacacac

SEQ ID NO: 189 - DNA, 39 bp, Artificial Sequence
  Description of Artificial Sequence: Synthetic primer
atagctcttcagggaccatgtctgtctccttcctcatct

SEQ ID NO: 190 - DNA, 38 bp, Artificial Sequence
  Description of Artificial Sequence: Synthetic primer
atagctcttcagggaccatggactggacctggagvatc

SEQ ID NO: 191 - DNA, 38 bp, Artificial Sequence
  Description of Artificial Sequence: Synthetic primer
atagctcttcagggaccatggactggatttggaggrtc

SEQ ID NO: 192 - DNA, 38 bp, Artificial Sequence
  Description of Artificial Sequence: Synthetic primer
atagctcttcagggaccatggactgcacctggaggatc

SEQ ID NO: 193 - DNA, 38 bp, Artificial Sequence
  Description of Artificial Sequence: Synthetic primer
atagctcttcagggaccatggactggacctggaggktc

SEQ ID NO: 194 - DNA, 38 bp, Artificial Sequence
  Description of Artificial Sequence: Synthetic primer
atagctcttcagggaccatggagttkggrctgagctgg

SEQ ID NO: 195 - DNA, 38 bp, Artificial Sequence
  Description of Artificial Sequence: Synthetic primer
atagctcttcagggaccatggagtttkggctkagctgg

SEQ ID NO: 196 - DNA, 38 bp, Artificial Sequence
  Description of Artificial Sequence: Synthetic primer
atagctcttcagggaccatggaactggggctccgctgg

SEQ ID NO: 197 - DNA, 38 bp, Artificial Sequence
  Description of Artificial Sequence: Synthetic primer
atagctcttcagggaccatggarttggggctgwgctgg

SEQ ID NO: 198 - DNA, 38 bp, Artificial Sequence
  Description of Artificial Sequence: Synthetic primer
atagctcttcagggaccatggggtcaaccgccatcctc

SEQ ID NO: 199 - DNA, 44 bp, Artificial Sequence
  Description of Artificial Sequence: Synthetic primer
atagctcttcagggaccatggacatgagggtsccygctcagctc

SEQ ID NO: 200 - DNA, 44 bp, Artificial Sequence
  Description of Artificial Sequence: Synthetic primer
atagctcttcagggaccatggacatgagrgtcctcgctcagctc

SEQ ID NO: 201 - DNA, 41 bp, Artificial Sequence
  Description of Artificial Sequence: Synthetic primer
atagctcttcagggaccatggaagccccagcdcagcttctc

SEQ ID NO: 202 - DNA, 41 bp, Artificial Sequence
  Description of Artificial Sequence: Synthetic primer
atagctcttcagggaccatggaaaccccagcgcagcttctc

SEQ ID NO: 203 - DNA, 41 bp, Artificial Sequence
  Description of Artificial Sequence: Synthetic primer
atagctcttcagggaccatggtgttgcagacccaggtcttc

SEQ ID NO: 204 - DNA, 41 bp, Artificial Sequence
  Description of Artificial Sequence: Synthetic primer
atagctcttcagggaccatggggtcccaggttcacctcctc

SEQ ID NO: 205 - DNA, 41 bp, Artificial Sequence
  Description of Artificial Sequence: Synthetic primer
atagctcttcagggaccatgaggctccytgctcagctcctg

SEQ ID NO: 206 - DNA, 33 bp, Artificial Sequence
  Description of Artificial Sequence: Synthetic primer
atagctcttcttcgtttgatctccascttggtc

SEQ ID NO: 207 - DNA, 33 bp, Artificial Sequence
  Description of Artificial Sequence: Synthetic primer
atagctcttcttcgtttaatctccagtcgtgtc

SEQ ID NO: 208 - DNA, 30 bp, Artificial Sequence
  Description of Artificial Sequence: Synthetic primer
atagctcttctggctgaggagacggtgacc

SEQ ID NO: 209 - DNA, 34 bp, Artificial Sequence
  Description of Artificial Sequence: Synthetic primer
atagctcttcatgtgacgctgttgtgactcagga

SEQ ID NO: 210 - DNA, 34 bp, Artificial Sequence
  Description of Artificial Sequence: Synthetic primer
atagctcttcatgtgaccytgtgctcactcagtc

SEQ ID NO: 211 - DNA, 37 bp, Artificial Sequence
  Description of Artificial Sequence: Synthetic primer
gatgctcttctgggctggcctaggacagtcamcytgg

SEQ ID NO: 212 - protein, 120 aa, Artificial Sequence
  Description of Artificial Sequence: Synthetic polypeptide
QVQLQESGPGLVKPSETLSLTCAVSGYSISSGYYWGWIRQPPGKGLEWIGSIYHSGTTYYNPSLKSRVTISVDTSKNQFSLKLNSVTAADTAVYYCATYSSGWYFYFDYWGQGTLVTVSS

SEQ ID NO: 213 - protein, 11 aa, Artificial Sequence
  Description of Artificial Sequence: Synthetic peptide
GYSISSGYYWG

SEQ ID NO: 214 - protein, 16 aa, Artificial Sequence
  Description of Artificial Sequence: Synthetic peptide
SIYHSGTTYYNPSLKS

SEQ ID NO: 215 - protein, 11 aa, Artificial Sequence
  Description of Artificial Sequence: Synthetic peptide
YSSGWYFYFDY

SEQ ID NO: 216 - protein, 107 aa, Artificial Sequence
  Description of Artificial Sequence: Synthetic polypeptide
DIQLTQSPSFLSASVGDRVTITCRASQGISSYLAWYQQKPGKAPKLLIYVASTLQSGVPSRFSGSGSGTEFTLTISSLQPEDFATYYCQQLNSYPITFGQGTRLEIK

SEQ ID NO: 217 - protein, 11 aa, Artificial Sequence
  Description of Artificial Sequence: Synthetic peptide
RASQGISSYLA

SEQ ID NO: 218 - protein, 7 aa, Artificial Sequence
  Description of Artificial Sequence: Synthetic peptide
VASTLQS

SEQ ID NO: 219 - protein, 9 aa, Artificial Sequence
  Description of Artificial Sequence: Synthetic peptide
QQLNSYPIT

SEQ ID NO: 220 - protein, 119 aa, Artificial Sequence
  Description of Artificial Sequence: Synthetic polypeptide
QVQLVESGGGVVQPGRSLRLSCAVSGFSLTSYGVQWVRQAPGKGLEWLGVIWSSGSTDYNAAFLSRLTISKDNSKNTVYFQMNSLRAEDTAVYYCARDVTTIVEGFAHWGQGTLVTVSS

SEQ ID NO: 221 - protein, 10 aa, Artificial Sequence
  Description of Artificial Sequence: Synthetic peptide
GFSLTSYGVQ

SEQ ID NO: 222 - protein, 16 aa, Artificial Sequence
  Description of Artificial Sequence: Synthetic peptide
VIWSSGSTDYNAAFLS

SEQ ID NO: 223 - protein, 11 aa, Artificial Sequence
  Description of Artificial Sequence: Synthetic peptide
DVTTIVEGFAH

SEQ ID NO: 224 - protein, 107 aa, Artificial Sequence
  Description of Artificial Sequence: Synthetic polypeptide
DIQMTQSPSSLSASVGDRVTITCKASEKVGTYVSWYQQKPGKAPKLLIYGASNRYTGVPSRFSGSGSGTDFTLTISSLQPEDFATYYCGQTYSYPFTFGQGTKLEIK

SEQ ID NO: 225 - protein, 11 aa, Artificial Sequence
  Description of Artificial Sequence: Synthetic peptide
KASEKVGTYVS

SEQ ID NO: 226 - protein, 7 aa, Artificial Sequence
  Description of Artificial Sequence: Synthetic peptide
GASNRYT

SEQ ID NO: 227 - protein, 9 aa, Artificial Sequence
  Description of Artificial Sequence: Synthetic peptide
GQTYSYPFT

SEQ ID NO: 228 - protein, 119 aa, Artificial Sequence
  Description of Artificial Sequence: Synthetic polypeptide
QVQLVESGPGVVQPGRSLRLSCAVSGFSLTSYGVQWVRQAPGKGLEWLAVIWSSGSTDYNAAFLSRLTISKDNSKSTVYFQMNSLRAEDTAVYYCARDVTTIVEGFAHWGQGTLVTVSS

SEQ ID NO: 229 - protein, 10 aa, Artificial Sequence
  Description of Artificial Sequence: Synthetic peptide
GFSLTSYGVQ

SEQ ID NO: 230 - protein, 16 aa, Artificial Sequence
  Description of Artificial Sequence: Synthetic peptide
VIWSSGSTDYNAAFLS

SEQ ID NO: 231 - protein, 11 aa, Artificial Sequence
  Description of Artificial Sequence: Synthetic peptide
DVTTIVEGFAH

SEQ ID NO: 232 - protein, 119 aa, Artificial Sequence
  Description of Artificial Sequence: Synthetic polypeptide
QVQLVESGGGVVQPGRSLRLSCAVSGFSLTSYGVQWVRQAPGKGLEWLAVIWSSGSTDYNAAFLSRLTISKDNSKNTVYFQMNSLRAEDTAVYYCARDVTTIVEGFAHWGQGTLVTVSS

SEQ ID NO: 233 - protein, 10 aa, Artificial Sequence
  Description of Artificial Sequence: Synthetic peptide
GFSLTSYGVQ

SEQ ID NO: 234 - protein, 16 aa, Artificial Sequence
  Description of Artificial Sequence: Synthetic peptide
VIWSSGSTDYNAAFLS

SEQ ID NO: 235 - protein, 11 aa, Artificial Sequence
  Description of Artificial Sequence: Synthetic peptide
DVTTIVEGFAH

SEQ ID NO: 236 - protein, 119 aa, Artificial Sequence
  Description of Artificial Sequence: Synthetic polypeptide
QVQLVESGGGVVQPGRSLRLSCAVSGFTFSSYGVQWVRQAPGKGLEWLGVIWSSGSTDYNAAFLSRLTISKDNSKNTVYFQMNSLRAEDTAVYYCARDVTTIVEGFAHWGQGTLVTVSS

SEQ ID NO: 237 - protein, 10 aa, Artificial Sequence
  Description of Artificial Sequence: Synthetic peptide
GFTFSSYGVQ

SEQ ID NO: 238 - protein, 16 aa, Artificial Sequence
  Description of Artificial Sequence: Synthetic peptide
VIWSSGSTDYNAAFLS

SEQ ID NO: 239 - protein, 11 aa, Artificial Sequence
  Description of Artificial Sequence: Synthetic peptide
DVTTIVEGFAH

SEQ ID NO: 240 - protein, 119 aa, Artificial Sequence
  Description of Artificial Sequence: Synthetic polypeptide
EVQLVESGGGLVQPGGSLRLSCAVSGFSLTSYGVQWVRQAPGKGLEWLGVIWSSGSTDYNAAFLSRLTISKDTSKNTVYFQMNSLRAEDTAVYYCARDVTTIVEGFAHWGQGTLVTVSS

SEQ ID NO: 241 - protein, 10 aa, Artificial Sequence
  Description of Artificial Sequence: Synthetic peptide
GFSLTSYGVQ

SEQ ID NO: 242 - protein, 16 aa, Artificial Sequence
  Description of Artificial Sequence: Synthetic peptide
VIWSSGSTDYNAAFLS

SEQ ID NO: 243 - protein, 11 aa, Artificial Sequence
  Description of Artificial Sequence: Synthetic peptide
DVTTIVEGFAH

SEQ ID NO: 244 - protein, 107 aa, Artificial Sequence
  Description of Artificial Sequence: Synthetic polypeptide
DIQMTQSPSSLSASVGDRVTITCKASEKVGTYVSWYQQKPGKAPKLLIYGASNRYTGVPSRFSGSRSGTDFTLTISSLQPEDFATYYCGQTYSYPFTFGQGTKVEIK

SEQ ID NO: 245 - protein, 11 aa, Artificial Sequence
  Description of Artificial Sequence: Synthetic peptide
KASEKVGTYVS

SEQ ID NO: 246 - protein, 7 aa, Artificial Sequence
  Description of Artificial Sequence: Synthetic peptide
GASNRYT

SEQ ID NO: 247 - protein, 9 aa, Artificial Sequence
  Description of Artificial Sequence: Synthetic peptide
GQTYSYPFT

SEQ ID NO: 248 - protein, 123 aa, Artificial Sequence
  Description of Artificial Sequence: Synthetic polypeptide
QVQLQESGPGLVKPSGTLSLTCAVSGGSISSSNWWSWVRQPPGKGLEAIGEIYHSGNTNYNPSLKSRVTISVDKSKNQFSLKLSSVTAADTAIYYCARDGYSSGWYWGYFDYWGQGTLVTVSS

SEQ ID NO: 249 - protein, 11 aa, Artificial Sequence
  Description of Artificial Sequence: Synthetic peptide
GGSISSSNWWS

SEQ ID NO: 250 - protein, 16 aa, Artificial Sequence
  Description of Artificial Sequence: Synthetic peptide
EIYHSGNTNYNPSLKS

SEQ ID NO: 251 - protein, 8 aa, Artificial Sequence
  Description of Artificial Sequence: Synthetic peptide
DGYSSGWY

SEQ ID NO: 252 - protein, 107 aa, Artificial Sequence
  Description of Artificial Sequence: Synthetic polypeptide
EIVMTQSPATLSVSPGERATLSCRASQSVNSNLAWYQQKPGQAPWLLIYGASTRATGIPARFSGSGSGTEFTLTISSLQSEDFAVYYCQQYNHWPYTFGQGTKLEIK

SEQ ID NO: 253 - protein, 11 aa, Artificial Sequence
  Description of Artificial Sequence: Synthetic peptide
RASQSVNSNLA

SEQ ID NO: 254 - protein, 7 aa, Artificial Sequence
  Description of Artificial Sequence: Synthetic peptide
GASTRAT

SEQ ID NO: 255 - protein, 9 aa, Artificial Sequence
  Description of Artificial Sequence: Synthetic peptide
QQYNHWPYT

SEQ ID NO: 256 - protein, 123 aa, Artificial Sequence
  Description of Artificial Sequence: Synthetic polypeptide
QVQLQESGPGLVKPSETLSLTCTVSGGSISHYYWSWIRQPPGKGLEWIGYIYYSGPTNYNPSLKSRVTISVDTSKNQFSLKLSSVTAADTAVYYCARTYYYGSGSFPDAFDIWGQGTMVTVSS

SEQ ID NO: 257 - protein, 10 aa, Artificial Sequence
  Description of Artificial Sequence: Synthetic peptide
GGSISHYYWS

SEQ ID NO: 258 - protein, 16 aa, Artificial Sequence
  Description of Artificial Sequence: Synthetic peptide
YIYYSGPTNYNPSLKS

SEQ ID NO: 259 - protein, 15 aa, Artificial Sequence
  Description of Artificial Sequence: Synthetic peptide
TYYYGSGSFPDAFDI

SEQ ID NO: 260 - protein, 107 aa, Artificial Sequence
  Description of Artificial Sequence: Synthetic polypeptide
KIVLTQSPATLSLSPGERATLSCRASQSVSSYLAWYQQTPGQAPRLLIYDASNRATGIPARFSVSGSGTDFTLTISSLEPEDFAVYYCQQRSSWPLTFGGGTKLEIK

SEQ ID NO: 261 - protein, 11 aa, Artificial Sequence
  Description of Artificial Sequence: Synthetic peptide
RASQSVSSYLA

SEQ ID NO: 262 - protein, 7 aa, Artificial Sequence
  Description of Artificial Sequence: Synthetic peptide
DASNRAT

SEQ ID NO: 263 - protein, 9 aa, Artificial Sequence
  Description of Artificial Sequence: Synthetic peptide
QQRSSWPLT

SEQ ID NO: 264 - protein, 116 aa, Artificial Sequence
  Description of Artificial Sequence: Synthetic polypeptide
QVQLVQSGAEVKKPGSSMKVSCKASGDTFSSYAISWVRQAPGQGLEWMAGIIPVFGTAHNAQKFQGRVTITADKSTSTAYMELSSLRSEDTAVYYCTRGGPYFDYWGQGTLVTVSS

SEQ ID NO: 265 - protein, 10 aa, Artificial Sequence
  Description of Artificial Sequence: Synthetic peptide
GDTFSSYAIS

SEQ ID NO: 266 - protein, 17 aa, Artificial Sequence
  Description of Artificial Sequence: Synthetic peptide
GIIPVFGTAHNAQKFQG

SEQ ID NO: 267 - protein, 7 aa, Artificial Sequence
  Description of Artificial Sequence: Synthetic peptide
GGPYFDY

SEQ ID NO: 268 - protein, 107 aa, Artificial Sequence
  Description of Artificial Sequence: Synthetic polypeptide
EIVMTQSPATLSVSPGERAALSCRASQSVSSNLAWYQQKPGQAPRLLIYGVSTRATGIPDRFNGSGSGTEFTLTISSLQSEDFGAYYCQQYKKWPFIFGPGTKLEIK

SEQ ID NO: 269 - protein, 11 aa, Artificial Sequence
  Description of Artificial Sequence: Synthetic peptide
RASQSVSSNLA

SEQ ID NO: 270 - protein, 7 aa, Artificial Sequence
  Description of Artificial Sequence: Synthetic peptide
GVSTRAT

SEQ ID NO: 271 - protein, 9 aa, Artificial Sequence
  Description of Artificial Sequence: Synthetic peptide
QQYKKWPFI

SEQ ID NO: 272 - protein, 119 aa, Artificial Sequence
  Description of Artificial Sequence: Synthetic polypeptide
QVQLQESGPGLVKPSETLSLTCTVSGGSISSYYWSWIRQPPGKGLEWIGYIYYSGSTNNNPSLKSRVTISVDTSKNQFSLKLISVTAADTAVYYCARVYNNYDWGFDYWGQGTLVTVSS

SEQ ID NO: 273 - protein, 10 aa, Artificial Sequence
  Description of Artificial Sequence: Synthetic peptide
GGSISSYYWS

SEQ ID NO: 274 - protein, 16 aa, Artificial Sequence
  Description of Artificial Sequence: Synthetic peptide
YIYYSGSTNNNPSLKS

SEQ ID NO: 275 - protein, 11 aa, Artificial Sequence
  Description of Artificial Sequence: Synthetic peptide
VYNNYDWGFDY

SEQ ID NO: 276 - protein, 107 aa, Artificial Sequence
  Description of Artificial Sequence: Synthetic polypeptide
EIVMTQSPATLSVSPGERATLSCRASQSVSSNLAWYQQKPGQAPRLLIYGASTRATGIPARFSGSGSGTEFTLTIRSLQSEDFAVYYCQQYHNWPLTFGGGTKLEIK

SEQ ID NO: 277 - protein, 9 aa, Artificial Sequence
  Description of Artificial Sequence: Synthetic peptide
QQYHNWPLT

SEQ ID NO: 278 - protein, 116 aa, Artificial Sequence
  Description of Artificial Sequence: Synthetic polypeptide
QVQLVHSGAEVKRPGSSVKVSCKASGGTFSSYAISWVRQAPGQGLEWMGGIIPIFGIANYAQKFQGRVTIIADKSTRTAYMELSSLRSEDTAVYYCARGGPYFDYWGQGILVTVSS

SEQ ID NO: 279 - protein, 10 aa, Artificial Sequence
  Description of Artificial Sequence: Synthetic peptide
GGTFSSYAIS

SEQ ID NO: 280 - protein, 17 aa, Artificial Sequence
  Description of Artificial Sequence: Synthetic peptide
GIIPIFGIANYAQKFQG

SEQ ID NO: 281 - protein, 107 aa, Artificial Sequence
  Description of Artificial Sequence: Synthetic polypeptide
EIVMTQSPATLSVSPGERATLSCRASQSVSSNLAWYQQKPGQAPRLLIYGASTRATGIPARFSGSGSGTEFTLTISSLQSEDFAVYYCQQYNKWPFTFGPGTKVDIK

SEQ ID NO: 282 - protein, 9 aa, Artificial Sequence
  Description of Artificial Sequence: Synthetic peptide
QQYNKWPFT

SEQ ID NO: 283 - protein, 116 aa, Artificial Sequence
  Description of Artificial Sequence: Synthetic polypeptide
QVQVVQSGAEVKKPGSSVKVSCKASGDTFSNYAISWVRQAPGQGLEWMGGIIPIFGITNYAQKFQGRVTIIADKSTRTAYMELSSLRSEDTAVYYCSRGGPYFDYWGQGILVTVSS

SEQ ID NO: 284 - protein, 10 aa, Artificial Sequence
  Description of Artificial Sequence: Synthetic peptide
GDTFSNYAIS

SEQ ID NO: 285 - protein, 17 aa, Artificial Sequence
  Description of Artificial Sequence: Synthetic peptide
GIIPIFGITNYAQKFQG

SEQ ID NO: 286 - protein, 107 aa, Artificial Sequence
  Description of Artificial Sequence: Synthetic polypeptide
EIVMTQSPATLSVSPGERATLSCRASQSVSSNLAWYQQKPGQAPRLLIYGASTRATGIPARFSGSGSGTEFTLTISSLQSEDFAVYYCQQYKKWPFTFGPGTKVDIK

SEQ ID NO: 287 - protein, 9 aa, Artificial Sequence
  Description of Artificial Sequence: Synthetic peptide
QQYKKWPFT

SEQ ID NO: 288 - DNA, 360 bp, Artificial Sequence
  Description of Artificial Sequence: Synthetic polynucleotide
caggtgcagctgcaggagtcgggcccaggactggtgaagccttcggagaccctgtccctcacctgcgctgtctctggttactccatcagtagtggttattactggggctggatccggcagcccccaggaaaggggctggagtggattgggagtatctatcatagtgggaccacctactacaatccgtccctcaagagtcgagtcaccatatcagtggacacgtccaagaaccagttctccctgaagctgaactctgtgaccgccgcagacacggccgtgtattactgtgcgacctatagcagtggctggtacttctactttgactactggggccagggaaccctggtcaccgtctcctca

SEQ ID NO: 289 - DNA, 321 bp, Artificial Sequence
  Description of Artificial Sequence: Synthetic polynucleotide
gacatccagttgacccagtctccatccttcctgtctgcatctgtaggagacagagtcaccatcacttgccgggccagtcagggcattagcagttatttagcctggtatcagcaaaaaccagggaaagcccctaagctcctgatctatgttgcatccactttgcaaagtggggtcccatcaaggttcagcggcagtggatctgggacagaattcactctcacaatcagcagcctgcagcctgaagattttgcaacttattactgtcaacagcttaatagttacccgatcaccttcggccaagggacacgactggagattaaa

SEQ ID NO: 290 - DNA, 357 bp, Artificial Sequence
  Description of Artificial Sequence: Synthetic polynucleotide
caagttcaactcgtggaatccggtggcggggtagtacaacctggtcgcagcctccggctttcatgcgctgttagtggtttctctctcacatcttacggtgtgcaatgggtacggcaagcccccggcaagggtttggaatggctcggagtgatctggagtagcgggtctaccgactataacgctgcgtttcttagcaggctgactatttctaaagataattccaaaaatacggtttatttccaaatgaactccctgcgggctgaagacactgccgtttattactgtgctcgggatgttacaacgattgtagaaggcttcgcccattggggccaagggacattggtcacagtatcctca

SEQ ID NO: 291 - DNA, 321 bp, Artificial Sequence
  Description of Artificial Sequence: Synthetic polynucleotide
gacattcagatgacccaatcacctagttcactctcagcaagtgtaggtgacagagtaacaattacatgcaaggccagcgaaaaagttggcacctacgtgagttggtaccagcaaaaaccgggcaaagctccgaaattgcttatttacggtgcttcaaatcgctatactggagtgcccagtcgatttagtgggtctggctcaggtaccgactttacactcaccatctctagcctgcagccagaggactttgcgacgtattattgcggccagacgtatagttatccgttcacctttggacaaggtaccaagttggaaataaag

SEQ ID NO: 292 - DNA, 357 bp, Artificial Sequence
  Description of Artificial Sequence: Synthetic polynucleotide
caagtccagttggttgagagcggtcctggggtcgtgcagcctgggcggtctctgaggctgagttgtgcagtgtcaggtttcagccttacatcatacggggttcaatgggtaaggcaagcacctgggaaaggtctggaatggcttgcggtaatttggtctagcggtagcactgactacaatgcggcgtttctgagtaggctcacgatttctaaagacaattcaaaaagcacggtttattttcaaatgaacagtcttcgagcagaagatactgctgtttactattgtgctcgcgacgtgacgacaatcgtggagggattcgcccattggggtcagggcaccctcgttactgtaagttct

SEQ ID NO: 293 - DNA, 357 bp, Artificial Sequence
  Description of Artificial Sequence: Synthetic polynucleotide
caggttcaacttgtagagtctggtggtggagttgtgcaaccgggtaggtccctccgcctctcatgcgcagtgtctgggttctccttgactagctacggggttcagtgggtccggcaagccccaggaaagggtcttgaatggttggcagtaatttggtccagcggaagtaccgattataacgcagccttcctgtcccggttgaccataagtaaggataattcaaaaaacaccgtttactttcagatgaatagtctgcgagcggaggacacagcggtttactactgcgctagagacgttaccaccattgtggaagggtttgctcattggggtcaagggacacttgtgacggtttctagc

SEQ ID NO: 294 - DNA, 357 bp, Artificial Sequence
  Description of Artificial Sequence: Synthetic polynucleotide
caagttcaacttgttgagtcagggggaggagttgtgcaaccgggccgctccctgcgactttcatgtgcagtatcaggctttaccttttcatcctacggggtccaatgggttaggcaggctccaggtaaaggactggaatggcttggtgtaatatggagcagcggcagtacggattacaatgctgcattcttgagtcggctcactatatcaaaggacaactctaagaataccgtctattttcaaatgaactcactgcgcgccgaagacaccgcagtttactattgcgcccgagatgtcactacaatagtggagggttttgcacattggggccaaggaaccctcgtaactgtgtcctca

SEQ ID NO: 295 - DNA, 357 bp, Artificial Sequence
  Description of Artificial Sequence: Synthetic polynucleotide
gaggttcaactcgtggaatctggaggaggtttggttcagccaggcggttctctccgactgtcttgcgctgtaagtggatttagtctgacgtcctatggagtacagtgggtgcgccaagctcctgggaagggcttggaatggttgggggtgatctggtcttccggttctacagattacaatgcagcattcctctcacgcctgactataagtaaagatacttctaaaaataccgtctactttcagatgaacagtcttagggctgaggatactgcggtctactattgtgcgagggatgtcacgacgattgtagaaggattcgctcactggggccagggcactttggtaacagtctcctca

SEQ ID NO: 296 - DNA, 321 bp, Artificial Sequence
  Description of Artificial Sequence: Synthetic polynucleotide
gacattcagatgactcaatctccttcatcccttagcgcatccgtaggagatcgagtgaccataacatgcaaggcctctgagaaagtagggacttacgtgagctggtatcagcaaaagccggggaaagcaccgaagttgctcatttatggggcgtctaataggtacacgggagtcccgagcagattttccggctctcggagtggaaccgactttacccttacaattagtagtctccaacctgaggattttgccacgtactactgtggccagacttactcttatccatttacattcggccaaggtacgaaggttgaaattaaa

SEQ ID NO: 297 - DNA, 369 bp, Artificial Sequence
  Description of Artificial Sequence: Synthetic polynucleotide
caggtgcagctgcaggagtcgggcccaggactggtgaagccttcggggaccctgtccctcacctgcgctgtctctggtggctccatcagcagtagtaactggtggagttgggtccgccagcccccagggaaggggctggaggccattggggaaatctatcatagtggaaacaccaactacaacccgtccctcaagagtcgagtcaccatatcagtagacaagtccaagaaccagttctccctgaagctgagctctgtgaccgccgcggacacggccatttattactgtgcgagagatgggtatagcagtggctggtactggggctactttgactactggggccagggaaccctggtcaccgtctcctca

SEQ ID NO: 298 - DNA, 321 bp, Artificial Sequence
  Description of Artificial Sequence: Synthetic polynucleotide
gaaatagtgatgacgcagtctccagccaccctgtctgtgtctccaggggaaagagccaccctctcctgcagggccagtcagagtgttaacagcaacttagcctggtaccagcagaaacctggccaggctccctggctcctcatctatggtgcatccaccagggccactggtatcccagccaggttcagtggcagtgggtctgggacagagttcactctcaccatcagcagcctgcagtctgaagattttgcagtttattactgtcagcagtataatcactggccgtacacttttggccaggggaccaagctggagatcaaa

SEQ ID NO: 299 - DNA, 369 bp, Artificial Sequence
  Description of Artificial Sequence: Synthetic polynucleotide
caggtgcagctgcaggagtcgggccccggactggtgaagccttcggagaccctgtccctcacctgcactgtctctggtggctccatcagtcattactactggagctggatccggcagcccccagggaagggactggagtggattgggtatatctattacagtgggcccaccaactacaacccctccctcaagagtcgagtcaccatatcagtagacacgtccaagaaccagttctccctgaagctgagctctgtgaccgctgcggacacggccgtgtattactgtgcgaggacgtattactatggttcggggagttttcccgatgcttttgatatctggggccaagggacaatggtcaccgtctcctca

SEQ ID NO: 300 - DNA, 321 bp, Artificial Sequence
  Description of Artificial Sequence: Synthetic polynucleotide
aaaattgtgttgacacagtctccagccaccctgtctttgtctccaggtgaaagagccaccctctcctgcagggccagtcagagtgttagcagctacttagcctggtaccaacagacacctggccaggctcccaggctcctcatctatgatgcatccaacagggccactggcatcccagccaggttcagtgtcagtgggtctgggacagacttcactctcaccatcagcagcctagagcctgaagattttgcagtttattactgtcagcagcgtagcagctggcctctcactttcggcggagggaccaagctggagatcaaa

SEQ ID NO: 301 - DNA, 348 bp, Artificial Sequence
  Description of Artificial Sequence: Synthetic polynucleotide
caggtgcagctggtgcagtctggggctgaggtgaagaagcctgggtcctcaatgaaggtctcctgcaaggcttctggagacaccttcagcagctatgctatcagctgggtgcgacaggcccctggacaagggcttgagtggatggcagggatcatccctgtctttggtacagcacacaacgcacagaagttccagggcagagtcacgattaccgcggacaaatccacgagcacagcctacatggagctgagcagcctgagatctgaggacacggccgtgtattactgtacgagagggggtccttactttgactactggggccagggaaccctggtcaccgtctcctca

SEQ ID NO: 302 - DNA, 321 bp, Artificial Sequence
  Description of Artificial Sequence: Synthetic polynucleotide
gaaatagtgatgacgcagtctccagccaccctgtctgtgtctccaggggaaagagccgccctctcctgtagggccagtcagagtgttagcagcaacttagcctggtaccagcagaaacctggccaggctcccaggctcctcatctatggtgtttctaccagggccactggtatcccagacaggttcaatggcagtgggtctgggacagagttcactctcaccatcagcagcctgcagtctgaagattttggagcttattactgtcagcagtataaaaagtggccattcattttcggccctgggaccaagctggagatcaaa

SEQ ID NO: 303 - DNA, 357 bp, Artificial Sequence
  Description of Artificial Sequence: Synthetic polynucleotide
caggtgcagctgcaggagtcgggcccaggactggtgaagccttcggagaccctgtccctcacctgcactgtctctggtggctccatcagtagttactactggagctggatccggcagcccccagggaagggactggagtggattgggtatatctattacagtgggagtaccaataacaacccctccctcaagagtcgagtcaccatatcagtagacacgtccaagaaccagttctccctgaagctgatctctgtgaccgctgcggacacggccgtatactactgtgcgagggtctataataattacgattggggctttgactactggggccagggaaccctggtcaccgtctcctca

SEQ ID NO: 304 - DNA, 321 bp, Artificial Sequence
  Description of Artificial Sequence: Synthetic polynucleotide
gaaatagtaatgacgcagtctccagccaccctgtctgtgtctccaggggagagagccaccctctcctgcagggccagtcagagtgttagcagcaacttagcctggtaccagcagaaacctggtcaggctcccagactcctcatctatggtgcatccaccagggccactggtatcccagccaggttcagtggcagtgggtctgggacagagttcactctcaccatccgcagcctgcagtctgaagattttgcagtttattactgtcagcagtatcataactggcctctcactttcggcggagggaccaagctggagatcaaa

SEQ ID NO: 305 - DNA, 348 bp, Artificial Sequence
  Description of Artificial Sequence: Synthetic polynucleotide
caggtgcagctggttcattctggggctgaggtgaagaggcctgggtcctcggtgaaggtctcctgcaaggcttctggaggcaccttcagcagctatgctatcagttgggtgcgacaggcccctggacaagggcttgagtggatgggagggatcatccctatctttggtatagcaaactacgcacagaagttccagggcagagtcacgattatcgcggacaaatccacgaggacagcctacatggagctgagcagcctgagatctgaggacacggccgtgtattactgtgcgagagggggtccttactttgactactggggccagggaatcctggtcaccgtctcctca

SEQ ID NO: 306 - DNA, 321 bp, Artificial Sequence
  Description of Artificial Sequence: Synthetic polynucleotide
gaaatagtgatgacgcagtctccagccaccctgtctgtgtctccaggggaaagagccaccctctcctgcagggccagtcagagtgttagcagcaacttagcctggtaccagcagaaacctggccaggctcccaggctcctcatctatggtgcatccaccagggccactggtatcccagccaggttcagtggcagtgggtctgggacagagttcactctcaccatcagcagcctgcagtctgaagattttgcagtttattactgtcagcagtataataagtggccattcactttcggccctgggaccaaagtggatatcaaa

SEQ ID NO: 307 - DNA, 348 bp, Artificial Sequence
  Description of Artificial Sequence: Synthetic polynucleotide
caggtgcaggtggtgcagtctggggctgaggtgaagaagcctgggtcctcggtgaaggtctcctgcaaggcttctggagacaccttcagcaactatgctatcagttgggtgcgacaggcccctggacaaggacttgagtggatgggagggatcatccctatctttggtataacaaactacgcacaaaagttccagggcagagtcacgattatcgcggacaaatccacgaggacagcctacatggagctgagcagcctgagatctgaggacacggccgtgtattactgttcgagagggggtccttactttgactactggggccagggaatcctggtcaccgtctcctca

SEQ ID NO: 308 - DNA, 321 bp, Artificial Sequence
  Description of Artificial Sequence: Synthetic polynucleotide
gaaatagtgatgacgcagtctccagccaccctgtctgtgtctccaggggaaagagccaccctctcctgcagggccagtcagagtgtgagcagcaacttagcctggtaccagcagaaacctggccaggctcccaggctcctcatctatggtgcatccaccagggccactggtatcccagccaggttcagtggcagtgggtctgggacagagttcactctcaccatcagcagcctgcagtctgaagattttgcagtttattactgtcagcagtataaaaagtggccattcactttcggccctgggaccaaagtggatatcaaa